European Patent Specification EP 3 736 291 B1, published August 16, 2023. Title: ANTI-FCRH5 ANTIBODIES. Applicant: GENENTECH, INC. Application DIVISIONAL APPLICATION OF EP 17198415.6. The sequence listing filed with the application follows.

SEQUENCE LISTING (136 sequences)

SEQ ID NO: 1 - protein, 977 aa, Homo sapiens
MLLWVILLVLAPVSGQFARTPRPIIFLQPPWTTVFQGERVTLTCKGFRFYSPQKTKWYHRYLGKEILRETPDNILEVQESGEYRCQAQGSPLSSPVHLDFSSASLILQAPLSVFEGDSVVLRCRAKAEVTLNNTIYKNDNVLAFLNKRTDFHIPHACLKDNGAYRCTGYKESCCPVSSNTVKIQVQEPFTRPVLRASSFQPISGNPVTLTCETQLSLERSDVPLRFRFFRDDQTLGLGWSLSPNFQITAMWSKDSGFYWCKAATMPYSVISDSPRSWIQVQIPASHPVLTLSPEKALNFEGTKVTLHCETQEDSLRTLYRFYHEGVPLRHKSVRCERGASISFSLTTENSGNYYCTADNGLGAKPSKAVSLSVTVPVSHPVLNLSSPEDLIFEGAKVTLHCEAQRGSLPILYQFHHEGAALERRSANSAGGVAISFSLTAEHSGNYYCTADNGFGPQRSKAVSLSVTVPVSHPVLTLSSAEALTFEGATVTLHCEVQRGSPQILYQFYHEDMPLWSSSTPSVGRVSFSFSLTEGHSGNYYCTADNGFGPQRSEVVSLFVTVPVSRPILTLRVPRAQAVVGDLLELHCEAPRGSPPILYWFYHEDVTLGSSSAPSGGEASFNLSLTAEHSGNYSCEANNGLVAQHSDTISLSVIVPVSRPILTFRAPRAQAVVGDLLELHCEALRGSSPILYWFYHEDVTLGKISAPSGGGASFNLSLTTEHSGIYSCEADNGLEAQRSEMVTLKVAVPVSRPVLTLRAPGTHAAVGDLLELHCEALRGSPLILYRFFHEDVTLGNRSSPSGGASLNLSLTAEHSGNYSCEADNGLGAQRSETVTLYITGLTANRSGPFATGVAGGLLSIAGLAAGALLLYCWLSRKAGRKPASDPARSPSDSDSQEPTYHNVPAWEELQPVYTNANPRGENVVYSEVRIIQEKKKHAVASDPRHLRNKGSPIIYSEVKVASTPVSGSLFLASSAPHR

SEQ ID NO: 2 - protein, 11 aa, Artificial Sequence
  source: /note="Description of Artificial Sequence: Synthetic peptide"
KASQNVITNVA

SEQ ID NO: 3 - protein, 11 aa, Artificial Sequence
  source: /note="Description of Artificial Sequence: Synthetic peptide"
KASQDVSNIVV

SEQ ID NO: 4 - protein, 11 aa, Artificial Sequence
  source: /note="Description of Artificial Sequence: Synthetic peptide"
RASQNIRNNLH

SEQ ID NO: 5 - protein, 11 aa, Artificial Sequence
  source: /note="Description of Artificial Sequence: Synthetic peptide"
RASQSISNNLH

SEQ ID NO: 6 - protein, 11 aa, Artificial Sequence
  source: /note="Description of Artificial Sequence: Synthetic peptide"
RASENIYSNLA

SEQ ID NO: 7 - protein, 16 aa, Artificial Sequence
  source: /note="Description of Artificial Sequence: Synthetic peptide"
RSSQSLVHRNGNTYLH

SEQ ID NO: 8 - protein, 11 aa, Artificial Sequence
  source: /note="Description of Artificial Sequence: Synthetic peptide"
RASENIYSNLA

SEQ ID NO: 9 - protein, 11 aa, Artificial Sequence
  source: /note="Description of Artificial Sequence: Synthetic peptide"
RASENIYSNLA

SEQ ID NO: 10 - protein, 11 aa, Artificial Sequence
  source: /note="Description of Artificial Sequence: Synthetic peptide"
RASQSISNNLH

SEQ ID NO: 11 - protein, 11 aa, Artificial Sequence
  source: /note="Description of Artificial Sequence: Synthetic peptide"
RASQNIRNNLH

SEQ ID NO: 12 - protein, 14 aa, Artificial Sequence
  source: /note="Description of Artificial Sequence: Synthetic peptide"
RSSTGTVTTSNFAN

SEQ ID NO: 13 - protein, 11 aa, Artificial Sequence
  source: /note="Description of Artificial Sequence: Synthetic peptide"
KASQDVGTAVA

SEQ ID NO: 14 - protein, 7 aa, Artificial Sequence
  source: /note="Description of Artificial Sequence: Synthetic peptide"
SASYRYS

SEQ ID NO: 15 - protein, 7 aa, Artificial Sequence
  source: /note="Description of Artificial Sequence: Synthetic peptide"
SASYRYT

SEQ ID NO: 16 - protein, 7 aa, Artificial Sequence
  source: /note="Description of Artificial Sequence: Synthetic peptide"
FTSQSIS

SEQ ID NO: 17 - protein, 7 aa, Artificial Sequence
  source: /note="Description of Artificial Sequence: Synthetic peptide"
FASQSIS

SEQ ID NO: 18 - protein, 7 aa, Artificial Sequence
  source: /note="Description of Artificial Sequence: Synthetic peptide"
GAANLAE

SEQ ID NO: 19 - protein, 7 aa, Artificial Sequence
  source: /note="Description of Artificial Sequence: Synthetic peptide"
KVSNRFS

SEQ ID NO: 20 - protein, 7 aa, Artificial Sequence
  source: /note="Description of Artificial Sequence: Synthetic peptide"
GAANLAE

SEQ ID NO: 21 - protein, 7 aa, Artificial Sequence
  source: /note="Description of Artificial Sequence: Synthetic peptide"
GAANLAE

SEQ ID NO: 22 - protein, 7 aa, Artificial Sequence
  source: /note="Description of Artificial Sequence: Synthetic peptide"
FASQSIS

SEQ ID NO: 23 - protein, 7 aa, Artificial Sequence
  source: /note="Description of Artificial Sequence: Synthetic peptide"
FASQSMS

SEQ ID NO: 24 - protein, 7 aa, Artificial Sequence
  source: /note="Description of Artificial Sequence: Synthetic peptide"
GTSNRAP

SEQ ID NO: 25 - protein, 7 aa, Artificial Sequence
  source: /note="Description of Artificial Sequence: Synthetic peptide"
WPSTRHT

SEQ ID NO: 26 - protein, 10 aa, Artificial Sequence
  source: /note="Description of Artificial Sequence: Synthetic peptide"
QQYTNYPMWT

SEQ ID NO: 27 - protein, 9 aa, Artificial Sequence
  source: /note="Description of Artificial Sequence: Synthetic peptide"
QQHYSSPYT

SEQ ID NO: 28 - protein, 10 aa, Artificial Sequence
  source: /note="Description of Artificial Sequence: Synthetic peptide"
QQSNNWPQYT

SEQ ID NO: 29 - protein, 10 aa, Artificial Sequence
  source: /note="Description of Artificial Sequence: Synthetic peptide"
QQSNNWPQYT

SEQ ID NO: 30 - protein, 9 aa, Artificial Sequence
  source: /note="Description of Artificial Sequence: Synthetic peptide"
QHFWGIPWT

SEQ ID NO: 31 - protein, 9 aa, Artificial Sequence
  source: /note="Description of Artificial Sequence: Synthetic peptide"
SQSTHVPPT

SEQ ID NO: 32 - protein, 9 aa, Artificial Sequence
  source: /note="Description of Artificial Sequence: Synthetic peptide"
QHFWGIPWT

SEQ ID NO: 33 - protein, 9 aa, Artificial Sequence
  source: /note="Description of Artificial Sequence: Synthetic peptide"
QHFWGIPWT

SEQ ID NO: 34 - protein, 10 aa, Artificial Sequence
  source: /note="Description of Artificial Sequence: Synthetic peptide"
QQSNNWPQYT

SEQ ID NO: 35 - protein, 10 aa, Artificial Sequence
  source: /note="Description of Artificial Sequence: Synthetic peptide"
QQSNNWPQYT

SEQ ID NO: 36 - protein, 9 aa, Artificial Sequence
  source: /note="Description of Artificial Sequence: Synthetic peptide"
VLWCSNLWV

SEQ ID NO: 37 - protein, 9 aa, Artificial Sequence
  source: /note="Description of Artificial Sequence: Synthetic peptide"
QQFSSLPHT

SEQ ID NO: 38 - protein, 5 aa, Artificial Sequence
  source: /note="Description of Artificial Sequence: Synthetic peptide"
AYIMN

SEQ ID NO: 39 - protein, 5 aa, Artificial Sequence
  source: /note="Description of Artificial Sequence: Synthetic peptide"
RFGVH

SEQ ID NO: 40 - protein, 5 aa, Artificial Sequence
  source: /note="Description of Artificial Sequence: Synthetic peptide"
DYYMK

SEQ ID NO: 41 - protein, 5 aa, Artificial Sequence
  source: /note="Description of Artificial Sequence: Synthetic peptide"
DYYMK

SEQ ID NO: 42 - protein, 5 aa, Artificial Sequence
  source: /note="Description of Artificial Sequence: Synthetic peptide"
EYTIH

SEQ ID NO: 43 - protein, 5 aa, Artificial Sequence
  source: /note="Description of Artificial Sequence: Synthetic peptide"
SYWIN

SEQ ID NO: 44 - protein, 5 aa, Artificial Sequence
  source: /note="Description of Artificial Sequence: Synthetic peptide"
EYTIH

SEQ ID NO: 45 - protein, 5 aa, Artificial Sequence
  source: /note="Description of Artificial Sequence: Synthetic peptide"
EYTIH

SEQ ID NO: 46 - protein, 5 aa, Artificial Sequence
  source: /note="Description of Artificial Sequence: Synthetic peptide"
DYYMK

SEQ ID NO: 47 - protein, 5 aa, Artificial Sequence
  source: /note="Description of Artificial Sequence: Synthetic peptide"
DYYMK

SEQ ID NO: 48 - protein, 5 aa, Artificial Sequence
  source: /note="Description of Artificial Sequence: Synthetic peptide"
NYLIE

SEQ ID NO: 49 - protein, 5 aa, Artificial Sequence
  source: /note="Description of Artificial Sequence: Synthetic peptide"
AYFMN

SEQ ID NO: 50 - protein, 10 aa, Artificial Sequence
  source: /note="Description of Artificial Sequence: Synthetic peptide"
GYSFTAYIMN

SEQ ID NO: 51 - protein, 10 aa, Artificial Sequence
  source: /note="Description of Artificial Sequence: Synthetic peptide"
GFSLTRFGVH

SEQ ID NO: 52 - protein, 10 aa, Artificial Sequence
  source: /note="Description of Artificial Sequence: Synthetic peptide"
GYTFTDYYMK

SEQ ID NO: 53 - protein, 10 aa, Artificial Sequence
  source: /note="Description of Artificial Sequence: Synthetic peptide"
GYTFTDYYMK

SEQ ID NO: 54 - protein, 10 aa, Artificial Sequence
  source: /note="Description of Artificial Sequence: Synthetic peptide"
GYTFTEYTIH

SEQ ID NO: 55 - protein, 10 aa, Artificial Sequence
  source: /note="Description of Artificial Sequence: Synthetic peptide"
GYTFISYWIN

SEQ ID NO: 56 - protein, 10 aa, Artificial Sequence
  source: /note="Description of Artificial Sequence: Synthetic peptide"
GYTFTEYTIH

SEQ ID NO: 57 - protein, 10 aa, Artificial Sequence
  source: /note="Description of Artificial Sequence: Synthetic peptide"
GYTFTEYTIH

SEQ ID NO: 58 - protein, 10 aa, Artificial Sequence
  source: /note="Description of Artificial Sequence: Synthetic peptide"
GYTFTDYYMK

SEQ ID NO: 59 - protein, 10 aa, Artificial Sequence
  source: /note="Description of Artificial Sequence: Synthetic peptide"
GYTFTDYYMK

SEQ ID NO: 60 - protein, 10 aa, Artificial Sequence
  source: /note="Description of Artificial Sequence: Synthetic peptide"
GYAFTNYLIE

SEQ ID NO: 61 - protein, 10 aa, Artificial Sequence
  source: /note="Description of Artificial Sequence: Synthetic peptide"
GFSFTAYFMN

SEQ ID NO: 62 - protein, 17 aa, Artificial Sequence
  source: /note="Description of Artificial Sequence: Synthetic peptide"
LINPYNGETTYNQKFKG

SEQ ID NO: 63 - protein, 16 aa, Artificial Sequence
  source: /note="Description of Artificial Sequence: Synthetic peptide"
VIWRGGSTDYNAAFMS

SEQ ID NO: 64 - protein, 17 aa, Artificial Sequence
  source: /note="Description of Artificial Sequence: Synthetic peptide"
DINPNNGETFYSQKFKG

SEQ ID NO: 65 - protein, 17 aa, Artificial Sequence
  source: /note="Description of Artificial Sequence: Synthetic peptide"
DINPYNGETFYNQKLKG

SEQ ID NO: 66 - protein, 17 aa, Artificial Sequence
  source: /note="Description of Artificial Sequence: Synthetic peptide"
GINPNNDAVSYNQRFRG

SEQ ID NO: 67 - protein, 17 aa, Artificial Sequence
  source: /note="Description of Artificial Sequence: Synthetic peptide"
NIYPSDSYTNYNQKFKD

SEQ ID NO: 68 - protein, 17 aa, Artificial Sequence
  source: /note="Description of Artificial Sequence: Synthetic peptide"
GINPNNDAISYNQKFRG

SEQ ID NO: 69 - protein, 17 aa, Artificial Sequence
  source: /note="Description of Artificial Sequence: Synthetic peptide"
GINPNNDAISYNQKFRG

SEQ ID NO: 70 - protein, 17 aa, Artificial Sequence
  source: /note="Description of Artificial Sequence: Synthetic peptide"
DINPYNGDTFYNQKFKD

SEQ ID NO: 71 - protein, 17 aa, Artificial Sequence
  source: /note="Description of Artificial Sequence: Synthetic peptide"
DINPNNGETFYNQKFKG

SEQ ID NO: 72 - protein, 17 aa, Artificial Sequence
  source: /note="Description of Artificial Sequence: Synthetic peptide"
VINPGSGGTNYNEKFKG

SEQ ID NO: 73 - protein, 17 aa, Artificial Sequence
  source: /note="Description of Artificial Sequence: Synthetic peptide"
RINPYNGETFFNQNFKD

SEQ ID NO: 74 - protein, 18 aa, Artificial Sequence
  source: /note="Description of Artificial Sequence: Synthetic peptide"
GLINPYNGETTYNQKFKG

SEQ ID NO: 75 - protein, 17 aa, Artificial Sequence
  source: /note="Description of Artificial Sequence: Synthetic peptide"
GVIWRGGSTDYNAAFMS

SEQ ID NO: 76 - protein, 18 aa, Artificial Sequence
  source: /note="Description of Artificial Sequence: Synthetic peptide"
GDINPNNGETFYSQKFKG

SEQ ID NO: 77 - protein, 18 aa, Artificial Sequence
  source: /note="Description of Artificial Sequence: Synthetic peptide"
GDINPYNGETFYNQKLKG

SEQ ID NO: 78 - protein, 18 aa, Artificial Sequence
  source: /note="Description of Artificial Sequence: Synthetic peptide"
GGINPNNDAVSYNQRFRG

SEQ ID NO: 79 - protein, 18 aa, Artificial Sequence
  source: /note="Description of Artificial Sequence: Synthetic peptide"
GNIYPSDSYTNYNQKFKD

SEQ ID NO: 80 - protein, 18 aa, Artificial Sequence
  source: /note="Description of Artificial Sequence: Synthetic peptide"
GGINPNNDAISYNQKFRG

SEQ ID NO: 81 - protein, 18 aa, Artificial Sequence
  source: /note="Description of Artificial Sequence: Synthetic peptide"
GGINPNNDAISYNQKFRG

SEQ ID NO: 82 - protein, 18 aa, Artificial Sequence
  source: /note="Description of Artificial Sequence: Synthetic peptide"
GDINPYNGDTFYNQKFKD

SEQ ID NO: 83 - protein, 18 aa, Artificial Sequence
  source: /note="Description of Artificial Sequence: Synthetic peptide"
GDINPNNGETFYNQKFKG

SEQ ID NO: 84 - protein, 18 aa, Artificial Sequence
  source: /note="Description of Artificial Sequence: Synthetic peptide"
GVINPGSGGTNYNEKFKG

SEQ ID NO: 85 - protein, 18 aa, Artificial Sequence
  source: /note="Description of Artificial Sequence: Synthetic peptide"
GRINPYNGETFFNQNFKD

SEQ ID NO: 86 - protein, 7 aa, Artificial Sequence
  source: /note="Description of Artificial Sequence: Synthetic peptide"
GLYWFPY

SEQ ID NO: 87 - protein, 12 aa, Artificial Sequence
  source: /note="Description of Artificial Sequence: Synthetic peptide"
HYYGSSDYALDN

SEQ ID NO: 88 - protein, 7 aa, Artificial Sequence
  source: /note="Description of Artificial Sequence: Synthetic peptide"
GLYRFDY

SEQ ID NO: 89 - protein, 7 aa, Artificial Sequence
  source: /note="Description of Artificial Sequence: Synthetic peptide"
GLYFFAY

SEQ ID NO: 90 - protein, 9 aa, Artificial Sequence
  source: /note="Description of Artificial Sequence: Synthetic peptide"
LGRGYYFDY

SEQ ID NO: 91 - protein, 12 aa, Artificial Sequence
  source: /note="Description of Artificial Sequence: Synthetic peptide"
SLYGYDASYFDY

SEQ ID NO: 92 - protein, 9 aa, Artificial Sequence
  source: /note="Description of Artificial Sequence: Synthetic peptide"
LGRGYYFDY

SEQ ID NO: 93 - protein, 9 aa, Artificial Sequence
  source: /note="Description of Artificial Sequence: Synthetic peptide"
LGRGYYFDY

SEQ ID NO: 94 - protein, 7 aa, Artificial Sequence
  source: /note="Description of Artificial Sequence: Synthetic peptide"
GLYFFHY

SEQ ID NO: 95 - protein, 7 aa, Artificial Sequence
  source: /note="Description of Artificial Sequence: Synthetic peptide"
GLYRFDY

SEQ ID NO: 96 - protein, 10 aa, Artificial Sequence
  source: /note="Description of Artificial Sequence: Synthetic peptide"
TRNYGYVIDY

SEQ ID NO: 97 - protein, 7 aa, Artificial Sequence
  source: /note="Description of Artificial Sequence: Synthetic peptide"
GLYYLNY

SEQ ID NO: 98 - protein, 9 aa, Artificial Sequence
  source: /note="Description of Artificial Sequence: Synthetic peptide"
ARGLYWFPY

SEQ ID NO: 99 - protein, 14 aa, Artificial Sequence
  source: /note="Description of Artificial Sequence: Synthetic peptide"
SNHYYGSSDYALDN

SEQ ID NO: 100 - protein, 9 aa, Artificial Sequence
  source: /note="Description of Artificial Sequence: Synthetic peptide"
ARGLYRFDY

SEQ ID NO: 101 - protein, 9 aa, Artificial Sequence
  source: /note="Description of Artificial Sequence: Synthetic peptide"
ARGLYFFAY

SEQ ID NO: 102 - protein, 11 aa, Artificial Sequence
  source: /note="Description of Artificial Sequence: Synthetic peptide"
AKLGRGYYFDY

SEQ ID NO: 103 - protein, 14 aa, Artificial Sequence
  source: /note="Description of Artificial Sequence: Synthetic peptide"
TRSLYGYDASYFDY

SEQ ID NO: 104 - protein, 11 aa, Artificial Sequence
  source: /note="Description of Artificial Sequence: Synthetic peptide"
AKLGRGYYFDY

SEQ ID NO: 105 - protein, 11 aa, Artificial Sequence
  source: /note="Description of Artificial Sequence: Synthetic peptide"
AKLGRGYYFDY

SEQ ID NO: 106 - protein, 9 aa, Artificial Sequence
  source: /note="Description of Artificial Sequence: Synthetic peptide"
ARGLYFFHY

SEQ ID NO: 107 - protein, 9 aa, Artificial Sequence
  source: /note="Description of Artificial Sequence: Synthetic peptide"
ARGLYRFDY

SEQ ID NO: 108 - protein, 12 aa, Artificial Sequence
  source: /note="Description of Artificial Sequence: Synthetic peptide"
ARTRNYGYVIDY

SEQ ID NO: 109 - protein, 9 aa, Artificial Sequence
  source: /note="Description of Artificial Sequence: Synthetic peptide"
GRGLYYLNY

SEQ ID NO: 110 - protein, 112 aa, Artificial Sequence
  source: /note="Description of Artificial Sequence: Synthetic polypeptide"
DIVMTQSQRFMSTSLGDRVSVTCKASQNVITNVAWYQQKPGQSPKALIYSASYRYSGVPDRFTGSGSGTDFTLTISNVQSEDLAEYFCQQYTNYPMWTFGGGTRLEIKRTVA

SEQ ID NO: 111 - protein, 129 aa, Artificial Sequence
  source: /note="Description of Artificial Sequence: Synthetic polypeptide"
EVQLQQSGPELVKPGASMKISCEASGYSFTAYIMNWVKQSRGKNLEWIGLINPYNGETTYNQKFKGKATLTVDQSSSTAYMELLSLTSEDSAVYFCARGLYWFPYWGQGTLVTVSAASTKGPSVFPLAP

SEQ ID NO: 112 - protein, 112 aa, Artificial Sequence
  source: /note="Description of Artificial Sequence: Synthetic polypeptide"
DIVMTQSHKIMSTSVGDRVSITCKASQDVSNIVVWFQQKPGQSPNLLIYSASYRYTGVPDRFTGSGSGTDFTFTISSVQAEDLAVYYCQQHYSSPYTFGGGTKLEIKRTVAA

SEQ ID NO: 113 - protein, 133 aa, Artificial Sequence
  source: /note="Description of Artificial Sequence: Synthetic polypeptide"
EVQLQESGPGLVQPSQSLSITCTVSGFSLTRFGVHWVRQSPGKGLEWLGVIWRGGSTDYNAAFMSRLTITKDNSKSQVFFKLNSLKVDDTAIYYCSNHYYGSSDYALDNWGQGTSVTVSSASTKGPSVFPLAP

SEQ ID NO: 114 - protein, 113 aa, Artificial Sequence
  source: /note="Description of Artificial Sequence: Synthetic polypeptide"
EIVLTQSPATLSVTPGDSVSLSCRASQNIRNNLHWYQQKSHESPRLLIKFTSQSISGIPSRFTGSGSGTDFTLSINSVETEDFGMYFCQQSNNWPQYTFGGGTKLEIKRTVAA

SEQ ID NO: 115 - protein, 129 aa, Artificial Sequence
  source: /note="Description of Artificial Sequence: Synthetic polypeptide"
EVQLQQSGPELWKPGASVKMSCKASGYTFTDYYMKWVKQTHGKSLEWIGDINPNNGETFYSQKFKGKATLTVDKSSTTAYMQLNSLTSEDSAVYYCARGLYRFDYWGQGTTLTVSSASTKGPSVFPLAP

SEQ ID NO: 116 - protein, 113 aa, Artificial Sequence
  source: /note="Description of Artificial Sequence: Synthetic polypeptide"
DIQMTQSPATLSVTPGDSVSLSCRASQSISNNLHWYQQKSHESPRLLIKFASQSISGIPSRFSGSGSGTDFTLSINSVETEDFGMYFCQQSNNWPQYTFGGGTKLELKRTVAA

SEQ ID NO: 117 - protein, 129 aa, Artificial Sequence
  source: /note="Description of Artificial Sequence: Synthetic polypeptide"
EVQLQQSGPELVKSGASVKMSCKASGYTFTDYYMKWVKQSHGKSLEWIGDINPYNGETFYNQKLKGKATLTVDKSSNTVFMQLNSLTSEDSAVYYCARGLYFFAYWGQGTTLTVSSASTKGPSVFPLAP

SEQ ID NO: 118 - protein, 112 aa, Artificial Sequence
  source: /note="Description of Artificial Sequence: Synthetic polypeptide"
DIQMTQSPASLSASVGETVTITCRASENIYSNLAWYQLKQGKSPQLLVYGAANLAEGVPSRISGSGSGTQYSLKINSLQSEDFGTYYCQHFWGIPWTFGGGTKLEIKRTVAA

SEQ ID NO: 119 - protein, 131 aa, Artificial Sequence
  source: /note="Description of Artificial Sequence: Synthetic polypeptide"
EVQLQQSGPELVKPGASVKISCKTSGYTFTEYTIHWVKQSHGKSLERIGGINPNNDAVSYNQRFRGKATLTVDKSSSTAYMELRSLTSEDSAVYYCAKLGRGYYFDYWGQGTTLTVSSASTKGPSVFPLAP

SEQ ID NO: 120 - protein, 117 aa, Artificial Sequence
  source: /note="Description of Artificial Sequence: Synthetic polypeptide"
DIQMTQTPLSLPVTLGDQASISCRSSQSLVHRNGNTYLHWYLQKPGQSPKLLIYKVSNRFSGVPDRFSGSGSGTDFTLKISRVEAEDLGVYFCSQSTHVPPTFGGGTKLELKRTVAA

SEQ ID NO: 121 - protein, 134 aa, Artificial Sequence
  source: /note="Description of Artificial Sequence: Synthetic polypeptide"
QVQLQQPGAELVRPGASVKLSCKTSGYTFISYWINWVKQRPGQGLEWIGNIYPSDSYTNYNQKFKDKATLTVDTSSSTAYMQLTSPTSEDSAVYYCTRSLYGYDASYFDYWGQGTTLTVSSASTKGPSVFPLAP

SEQ ID NO: 122 - protein, 112 aa, Artificial Sequence
  source: /note="Description of Artificial Sequence: Synthetic polypeptide"
DIVMTQSPASLSASVGETVTITCRASENIYSNLAWYQLKQGKSPQLLVYGAANLAEGVPSRISGSGSGTQYSLKINSLQSEDFGTYYCQHFWGIPWTFGGGTKLEIKRTVAA

SEQ ID NO: 123 - protein, 131 aa, Artificial Sequence
  source: /note="Description of Artificial Sequence: Synthetic polypeptide"
QVQLQQSGPELVKPGASVKISCKTSGYTFTEYTIHWVKQSHGKSLERIGGINPNNDAISYNQKFRGKATLTVDKSSSTAYMELRSLTSEDSAVYYCAKLGRGYYFDYWGRGTTLTVSSASTKGPSVFPLAP

SEQ ID NO: 124 - protein, 112 aa, Artificial Sequence; identical to SEQ ID NO: 122
  source: /note="Description of Artificial Sequence: Synthetic polypeptide"

SEQ ID NO: 125 - protein, 131 aa, Artificial Sequence
  source: /note="Description of Artificial Sequence: Synthetic polypeptide"
EVQLQQSGPELVKPGASVKISCKTSGYTFTEYTIHWVKQSHGKSLERIGGINPNNDAISYNQKFRGKATLTVDKSSSTAYMELRSLTSEDSAVYYCAKLGRGYYFDYWGRGTTLTVSSASTKGPSVFPLAP

SEQ ID NO: 126 - protein, 113 aa, Artificial Sequence
  source: /note="Description of Artificial Sequence: Synthetic polypeptide"
DIVLIQSPATLSVTLGGSVSLSCRASQSISNNLHWYQQKSHESPRLLIKFASQSISGIPSRFRGSGSGTDFTLTINSVETEDFGIYFCQQSNNWPQYTFGGGTKLELKRTVAA

SEQ ID NO: 127 - protein, 129 aa, Artificial Sequence
  source: /note="Description of Artificial Sequence: Synthetic polypeptide"
EVQLQQSGPELVKPGASVKMSCKASGYTFTDYYMKWVRQNHGKRLEWIGDINPYNGDTFYNQKFKDKATLTVDKSSSTAYMQFNSLTSEDSAVYYCARGLYFFHYWGQGTTLTVSSASTKGPSVFPLAP

SEQ ID NO: 128 - protein, 113 aa, Artificial Sequence
  source: /note="Description of Artificial Sequence: Synthetic polypeptide"
DIVLTQSPANLSVIPGDSVSLSCRASQNIRNNLHWYQQKSQESPRLLIKFASQSMSGTPSRFTGSGSGTDFTLTINTVETEDFGMYFCQQSNNWPQYTFGGGTKLEIKRTVAA

SEQ ID NO: 129 - protein, 130 aa, Artificial Sequence
  source: /note="Description of Artificial Sequence: Synthetic polypeptide"
EVQLQQSGPELWKPGASVKMSCKASGYTFTDYYMKWVKQSHGKSLEWIGDINPNNGETFYNQKFKGKATLTVDKSTSTAYMELNSLTTEDSAVYYCARGLYRFDYWGQGTTLTVSSAASTKGPSVFPLAP

SEQ ID NO: 130 - protein, 115 aa, Artificial Sequence
  source: /note="Description of Artificial Sequence: Synthetic polypeptide"
QAVVTQESALTTSPGETVTLTCRSSTGTVTTSNFANWVQEKPDHLFTGLIGGTSNRAPGVPARFSGSLIGDKAALTITGAQTEDEAIYFCVLWCSNLWVFGGGTKLTVLGQPKAA

SEQ ID NO: 131 - protein, 132 aa, Artificial Sequence
  source: /note="Description of Artificial Sequence: Synthetic polypeptide"
QVQLQQSGADLVRPGTSVKVSCKASGYAFTNYLIEWVKQRPGQGLEWIGVINPGSGGTNYNEKFKGKATLTADKSSSTAYMQLSSLTSDDSAVYFCARTRNYGYVIDYWGQGTTLTVSSASTKGPSVFPLAP

SEQ ID NO: 132 - protein, 112 aa, Artificial Sequence
  source: /note="Description of Artificial Sequence: Synthetic polypeptide"
DIVMTQSHKFMSTSVGDRVSITCKASQDVGTAVAWYQQKPGQSPKLLIFWPSTRHTGVPDRFTGSGSGTDFTLTIGNVQSEDLADYFCQQFSSLPHTFGGGTKLEIKRTVAA

SEQ ID NO: 133 - protein, 129 aa, Artificial Sequence
  source: /note="Description of Artificial Sequence: Synthetic polypeptide"
QVQLQQSGPELVKPGASVKISCKASGFSFTAYFMNWVKQSHGKSPEWIGRINPYNGETFFNQNFKDKATLTVDKSSNTAHMELLSLTSDDSAVYYCGRGLYYLNYWGQGTTLTVSSASTKGPSVFPLAP

SEQ ID NO: 134 - protein, 107 aa, Artificial Sequence
  source: /note="Description of Artificial Sequence: Synthetic polypeptide"
DIVMTQSHKIMSTSVGDRVSITCKASQDVSNIVVWFQQKPGQSPNLLIYSASYRYTGVPDRFTGSGSGTDFTFTISSVQAEDLAVYYCQQHYSSPYTFGGGTKLEIK

SEQ ID NO: 135 - protein, 120 aa, Artificial Sequence
  source: /note="Description of Artificial Sequence: Synthetic polypeptide"
QVQLKQSGPGLVQPSQSLSITCTVSGFSLTRFGVHWVRQSPGKGLEWLGVIWRGGSTDYNAAFMSRLTITKDNSKSQVFFKLNSLKVDDTAIYYCSNHYYGSSDYALDNWGQGISVTVSS

SEQ ID NO: 136 - protein, 233 aa, Homo sapiens
VAVPVSRPVLTLRAPGTHAAVGDLLELHCEALRGSPLILYRFFHEDVTLGNRSSPSGGASLNLSLTAEHSGNYSCEADNGLGAQRSETVTLYITGLTANRSGPFATGVAGGLLSIAGLAAGALLLYCWLSRKAGRKPASDPARSPSDSDSQEPTYHNVPAWEELQPVYTNANPRGENVVYSEVRIIQEKKKHAVASDPRHLRNKGSPIIYSEVKVASTPVSGSLFLASSAPHR